European Patent Application EP 4 574 838 A1, published June 25, 2025. Title: Chimeric antigen receptor (CAR) with enhanced recruitment of signalling partners. Applicant: Vilnius University. Application EP. The sequence listing filed with the application follows.

SEQUENCE LISTING (73 sequences)

SEQ ID NO: 1 - protein, 15 aa, synthetic construct
  REGION 1..15: note = linker
GGGGSGGGGSGGGGS

SEQ ID NO: 2 - protein, 120 aa, Mus musculus
  REGION 1..120: note = heavy chain variable region (VH)
EVKLQESGPGLVAPSQSLSVTCTVSGVSLPDYGVSWIRQPPRKGLEWLGVIWGSETTYYNSALKSRLTIIKDNSKSQVFLKMNSLQTDDTAIYYCAKHYYYGGSYAMDYWGQGTSVTVSS

SEQ ID NO: 3 - protein, 108 aa, Mus musculus
  REGION 1..108: note = light chain variable region (VL)
DIQMTQTTSSLSASLGDRVTISCRASQDISKYLNWYQQKPDGTVKLLIYHTSRLHSGVPSRFSGSGSGTDYSLTISNLEQEDIATYFCQQGNTLPYTFGGGTKLEITG

SEQ ID NO: 4 - protein, 243 aa, synthetic construct
  REGION 1..243: note = single chain variable fragment (scFv) in VL-VH configuration
DIQMTQTTSSLSASLGDRVTISCRASQDISKYLNWYQQKPDGTVKLLIYHTSRLHSGVPSRFSGSGSGTDYSLTISNLEQEDIATYFCQQGNTLPYTFGGGTKLEITGGGGGSGGGGSGGGGSEVKLQESGPGLVAPSQSLSVTCTVSGVSLPDYGVSWIRQPPRKGLEWLGVIWGSETTYYNSALKSRLTIIKDNSKSQVFLKMNSLQTDDTAIYYCAKHYYYGGSYAMDYWGQGTSVTVSS

SEQ ID NO: 5 - protein, 243 aa, synthetic construct
  REGION 1..243: note = single chain variable fragment (scFv) in VH-VL configuration
EVKLQESGPGLVAPSQSLSVTCTVSGVSLPDYGVSWIRQPPRKGLEWLGVIWGSETTYYNSALKSRLTIIKDNSKSQVFLKMNSLQTDDTAIYYCAKHYYYGGSYAMDYWGQGTSVTVSSGGGGSGGGGSGGGGSDIQMTQTTSSLSASLGDRVTISCRASQDISKYLNWYQQKPDGTVKLLIYHTSRLHSGVPSRFSGSGSGTDYSLTISNLEQEDIATYFCQQGNTLPYTFGGGTKLEITG

SEQ ID NO: 6 - protein, 174 aa, Homo sapiens
  REGION 1..174: note = Macrosialin Gp110 CD68
SPTSKETIGDYTWTNGSQPCVQPCVHLQAQIQIRVMYTTQGGGEAWGISVLNPNKTKVQGSCEGAHPHLLLSFPYGHLSFGFMQDLQQKVVYLSYMAVEYNVSFPHAAQWTFSAQNASLRDLQAPLGQSFSCSNSSIILSPAVHLDLLSLRLQAAQLPHTGVFGQSFSCPSDRS

SEQ ID NO: 7 - protein, 174 aa, synthetic construct
  REGION 1..174: note = CD68 ectodomain spacer
SPTSKETIGDYTWTNGSQPAVQPCVHLQAQIQIRVMYTTQGGGEAWGISVLNPNKTKVQGSCEGAHPHLLLSFPYGHLSFGFMQDLQQKVVYLSYMAVEYNVSFPHAAQWTFSAQNASLRDLQAPLGQSFSCSNSSIILSPAVHLDLLSLRLQAAQLPHTGVFGQSFSCPSDRS

SEQ ID NO: 8 - protein, 174 aa, synthetic construct
  REGION 1..174: note = CD68 ectodomain spacer
SPTSKETIGDYTWTNGSQPCVQPAVHLQAQIQIRVMYTTQGGGEAWGISVLNPNKTKVQGSCEGAHPHLLLSFPYGHLSFGFMQDLQQKVVYLSYMAVEYNVSFPHAAQWTFSAQNASLRDLQAPLGQSFSCSNSSIILSPAVHLDLLSLRLQAAQLPHTGVFGQSFSCPSDRS

SEQ ID NO: 9 - protein, 174 aa, synthetic construct
  REGION 1..174: note = CD68 ectodomain spacer
SPTSKETIGDYTWTNGSQPCVQPCVHLQAQIQIRVMYTTQGGGEAWGISVLNPNKTKVQGSAEGAHPHLLLSFPYGHLSFGFMQDLQQKVVYLSYMAVEYNVSFPHAAQWTFSAQNASLRDLQAPLGQSFSCSNSSIILSPAVHLDLLSLRLQAAQLPHTGVFGQSFSCPSDRS

SEQ ID NO: 10 - protein, 174 aa, synthetic construct
  REGION 1..174: note = CD68 ectodomain spacer
SPTSKETIGDYTWTNGSQPCVQPCVHLQAQIQIRVMYTTQGGGEAWGISVLNPNKTKVQGSCEGAHPHLLLSFPYGHLSFGFMQDLQQKVVYLSYMAVEYNVSFPHAAQWTFSAQNASLRDLQAPLGQSFSASNSSIILSPAVHLDLLSLRLQAAQLPHTGVFGQSFSCPSDRS

SEQ ID NO: 11 - protein, 174 aa, synthetic construct
  REGION 1..174: note = CD68 ectodomain spacer
SPTSKETIGDYTWTNGSQPCVQPCVHLQAQIQIRVMYTTQGGGEAWGISVLNPNKTKVQGSCEGAHPHLLLSFPYGHLSFGFMQDLQQKVVYLSYMAVEYNVSFPHAAQWTFSAQNASLRDLQAPLGQSFSCSNSSIILSPAVHLDLLSLRLQAAQLPHTGVFGQSFSAPSDRS

SEQ ID NO: 12 - protein, 174 aa, synthetic construct
  REGION 1..174: note = CD68 ectodomain spacer
SPTSKETIGDYTWTNGSQPAVQPAVHLQAQIQIRVMYTTQGGGEAWGISVLNPNKTKVQGSAEGAHPHLLLSFPYGHLSFGFMQDLQQKVVYLSYMAVEYNVSFPHAAQWTFSAQNASLRDLQAPLGQSFSASNSSIILSPAVHLDLLSLRLQAAQLPHTGVFGQSFSAPSDRS

SEQ ID NO: 13 - protein, 23 aa, Homo sapiens
  REGION 1..23: note = Glucose transporter type 4 (GLUT-4) transmembrane
AMGPYVFLLFAVLLLGFFIFTFL

SEQ ID NO: 14 - protein, 23 aa, synthetic construct
  REGION 1..23: note = Synthetic transmembrane peptide
ARGPYVFLLFAVLLLGFFIFTFL

SEQ ID NO: 15 - protein, 23 aa, synthetic construct
  REGION 1..23: note = Synthetic transmembrane peptide
AMRPYVFLLFAVLLLGFFIFTFL

SEQ ID NO: 16 - protein, 23 aa, synthetic construct
  REGION 1..23: note = Synthetic transmembrane peptide
AMGRYVFLLFAVLLLGFFIFTFL

SEQ ID NO: 17 - protein, 23 aa, synthetic construct
  REGION 1..23: note = Synthetic transmembrane peptide
AMGPRVFLLFAVLLLGFFIFTFL

SEQ ID NO: 18 - protein, 23 aa, synthetic construct
  REGION 1..23: note = Synthetic transmembrane peptide
AMGPYRFLLFAVLLLGFFIFTFL

SEQ ID NO: 19 - protein, 23 aa, synthetic construct
  REGION 1..23: note = Synthetic transmembrane peptide
AMGPYVRLLFAVLLLGFFIFTFL

SEQ ID NO: 20 - protein, 23 aa, synthetic construct
  REGION 1..23: note = Synthetic transmembrane peptide
AMGPYVFRLFAVLLLGFFIFTFL

SEQ ID NO: 21 - protein, 23 aa, synthetic construct
  REGION 1..23: note = Synthetic transmembrane peptide
AMGPYVFLRFAVLLLGFFIFTFL

SEQ ID NO: 22 - protein, 23 aa, synthetic construct
  REGION 1..23: note = Synthetic transmembrane peptide
AMGPYVFLLRAVLLLGFFIFTFL

SEQ ID NO: 23 - protein, 23 aa, synthetic construct
  REGION 1..23: note = Synthetic transmembrane peptide
AMGPYVFLLFRVLLLGFFIFTFL

SEQ ID NO: 24 - protein, 23 aa, synthetic construct
  REGION 1..23: note = Synthetic transmembrane peptide
AMGPYVFLLFARLLLGFFIFTFL

SEQ ID NO: 25 - protein, 23 aa, synthetic construct
  REGION 1..23: note = Synthetic transmembrane peptide
AMGPYVFLLFAVRLLGFFIFTFL

SEQ ID NO: 26 - protein, 23 aa, synthetic construct
  REGION 1..23: note = Synthetic transmembrane peptide
AMGPYVFLLFAVLRLGFFIFTFL

SEQ ID NO: 27 - protein, 23 aa, synthetic construct
  REGION 1..23: note = Synthetic transmembrane peptide
AMGPYVFLLFAVLLRGFFIFTFL

SEQ ID NO: 28 - protein, 23 aa, synthetic construct
  REGION 1..23: note = Synthetic transmembrane peptide
AMGPYVFLLFAVLLLRFFIFTFL

SEQ ID NO: 29 - protein, 23 aa, synthetic construct
  REGION 1..23: note = Synthetic transmembrane peptide
AMGPYVFLLFAVLLLGRFIFTFL

SEQ ID NO: 30 - protein, 23 aa, synthetic construct
  REGION 1..23: note = Synthetic transmembrane peptide
AMGPYVFLLFAVLLLGFRIFTFL

SEQ ID NO: 31 - protein, 23 aa, synthetic construct
  REGION 1..23: note = Synthetic transmembrane peptide
AMGPYVFLLFAVLLLGFFRFTFL

SEQ ID NO: 32 - protein, 23 aa, synthetic construct
  REGION 1..23: note = Synthetic transmembrane peptide
AMGPYVFLLFAVLLLGFFIRTFL

SEQ ID NO: 33 - protein, 23 aa, synthetic construct
  REGION 1..23: note = Synthetic transmembrane peptide
AMGPYVFLLFAVLLLGFFIFRFL

SEQ ID NO: 34 - protein, 23 aa, synthetic construct
  REGION 1..23: note = Synthetic transmembrane peptide
AMGPYVFLLFAVLLLGFFIFTRL

SEQ ID NO: 35 - protein, 23 aa, synthetic construct
  REGION 1..23: note = Synthetic transmembrane peptide
ARRPYVFLLFAVLLLGFFIFTFL

SEQ ID NO: 36 - protein, 23 aa, synthetic construct
  REGION 1..23: note = Synthetic transmembrane peptide
AMRRYVFLLFAVLLLGFFIFTFL

SEQ ID NO: 37 - protein, 23 aa, synthetic construct
  REGION 1..23: note = Synthetic transmembrane peptide
AMGRRVFLLFAVLLLGFFIFTFL

SEQ ID NO: 38 - protein, 23 aa, synthetic construct
  REGION 1..23: note = Synthetic transmembrane peptide
AMGPRRFLLFAVLLLGFFIFTFL

SEQ ID NO: 39 - protein, 23 aa, synthetic construct
  REGION 1..23: note = Synthetic transmembrane peptide
AMGPYRRLLFAVLLLGFFIFTFL

SEQ ID NO: 40 - protein, 23 aa, synthetic construct
  REGION 1..23: note = Synthetic transmembrane peptide
AMGPYVRRLFAVLLLGFFIFTFL

SEQ ID NO: 41 - protein, 23 aa, synthetic construct
  REGION 1..23: note = Synthetic transmembrane peptide
AMGPYVFRRFAVLLLGFFIFTFL

SEQ ID NO: 42 - protein, 23 aa, synthetic construct
  REGION 1..23: note = Synthetic transmembrane peptide
AMGPYVFLRRAVLLLGFFIFTFL

SEQ ID NO: 43 - protein, 23 aa, synthetic construct
  REGION 1..23: note = Synthetic transmembrane peptide
AMGPYVFLLRRVLLLGFFIFTFL

SEQ ID NO: 44 - protein, 23 aa, synthetic construct
  REGION 1..23: note = Synthetic transmembrane peptide
AMGPYVFLLFRRLLLGFFIFTFL

SEQ ID NO: 45 - protein, 23 aa, synthetic construct
  REGION 1..23: note = Synthetic transmembrane peptide
AMGPYVFLLFARRLLGFFIFTFL

SEQ ID NO: 46 - protein, 44 aa, Homo sapiens
  REGION 1..44: note = Glucose transporter type 4 (GLUT-4) endodomain
RVPETRGRTFDQISAAFRRTPSLLEQEVKPSTELEYLGPDENDG

SEQ ID NO: 47 - protein, 65 aa, Homo sapiens
  REGION 1..65: note = Glucose transporter type 4 (GLUT-4) endodomain
CPESPRYLYIIQNLEGPARKSLKRLTGWADVSGVLAELKDEKRKLERERPLSLLQLLGSRTHRQP

SEQ ID NO: 48 - protein, 109 aa, synthetic construct
  REGION 1..109: note = Synthetic Glucose transporter type 4 (GLUT-4) endodomain
CPESPRYLYIIQNLEGPARKSLKRLTGWADVSGVLAELKDEKRKLERERPLSLLQLLGSRTHRQPRVPETRGRTFDQISAAFRRTPSLLEQEVKPSTELEYLGPDENDG

SEQ ID NO: 49 - protein, 522 aa, synthetic construct
  REGION 1..522: note = Chimeric Antigen Receptor
MRPRLWLLLAAQLTVLHGNSVLEQKLISEEDLGGGGGGDIQMTQTTSSLSASLGDRVTISCRASQDISKYLNWYQQKPDGTVKLLIYHTSRLHSGVPSRFSGSGSGTDYSLTISNLEQEDIATYFCQQGNTLPYTFGGGTKLEITGGGGGSGGGGSGGGGSEVKLQESGPGLVAPSQSLSVTCTVSGVSLPDYGVSWIRQPPRKGLEWLGVIWGSETTYYNSALKSRLTIIKDNSKSQVFLKMNSLQTDDTAIYYCAKHYYYGGSYAMDYWGQGTSVTVSSSPTSKETIGDYTWTNGSQPAVQPAVHLQAQIQIRVMYTTQGGGEAWGISVLNPNKTKVQGSAEGAHPHLLLSFPYGHLSFGFMQDLQQKVVYLSYMAVEYNVSFPHAAQWTFSAQNASLRDLQAPLGQSFSASNSSIILSPAVHLDLLSLRLQAAQLPHTGVFGQSFSAPSDRSAMGPYVFLLFAVLLLGFFIFTFLRVPETRGRTFDQISAAFRRTPSLLEQEVKPSTELEYLGPDENDG

SEQ ID NO: 50 - protein, 522 aa, synthetic construct
  REGION 1..522: note = Chimeric Antigen Receptor
MRPRLWLLLAAQLTVLHGNSVLEQKLISEEDLGGGGGGDIQMTQTTSSLSASLGDRVTISCRASQDISKYLNWYQQKPDGTVKLLIYHTSRLHSGVPSRFSGSGSGTDYSLTISNLEQEDIATYFCQQGNTLPYTFGGGTKLEITGGGGGSGGGGSGGGGSEVKLQESGPGLVAPSQSLSVTCTVSGVSLPDYGVSWIRQPPRKGLEWLGVIWGSETTYYNSALKSRLTIIKDNSKSQVFLKMNSLQTDDTAIYYCAKHYYYGGSYAMDYWGQGTSVTVSSSPTSKETIGDYTWTNGSQPAVQPAVHLQAQIQIRVMYTTQGGGEAWGISVLNPNKTKVQGSAEGAHPHLLLSFPYGHLSFGFMQDLQQKVVYLSYMAVEYNVSFPHAAQWTFSAQNASLRDLQAPLGQSFSASNSSIILSPAVHLDLLSLRLQAAQLPHTGVFGQSFSAPSDRSAMGPRVFLLFAVLLLGFFIFTFLRVPETRGRTFDQISAAFRRTPSLLEQEVKPSTELEYLGPDENDG

SEQ ID NO: 51 - protein, 522 aa, synthetic construct
  REGION 1..522: note = Chimeric Antigen Receptor
MRPRLWLLLAAQLTVLHGNSVLEQKLISEEDLGGGGGGDIQMTQTTSSLSASLGDRVTISCRASQDISKYLNWYQQKPDGTVKLLIYHTSRLHSGVPSRFSGSGSGTDYSLTISNLEQEDIATYFCQQGNTLPYTFGGGTKLEITGGGGGSGGGGSGGGGSEVKLQESGPGLVAPSQSLSVTCTVSGVSLPDYGVSWIRQPPRKGLEWLGVIWGSETTYYNSALKSRLTIIKDNSKSQVFLKMNSLQTDDTAIYYCAKHYYYGGSYAMDYWGQGTSVTVSSSPTSKETIGDYTWTNGSQPAVQPAVHLQAQIQIRVMYTTQGGGEAWGISVLNPNKTKVQGSAEGAHPHLLLSFPYGHLSFGFMQDLQQKVVYLSYMAVEYNVSFPHAAQWTFSAQNASLRDLQAPLGQSFSASNSSIILSPAVHLDLLSLRLQAAQLPHTGVFGQSFSAPSDRSAMGPYRFLLFAVLLLGFFIFTFLRVPETRGRTFDQISAAFRRTPSLLEQEVKPSTELEYLGPDENDG

SEQ ID NO: 52 - protein, 522 aa, synthetic construct
  REGION 1..522: note = Chimeric Antigen Receptor
MRPRLWLLLAAQLTVLHGNSVLEQKLISEEDLGGGGGGDIQMTQTTSSLSASLGDRVTISCRASQDISKYLNWYQQKPDGTVKLLIYHTSRLHSGVPSRFSGSGSGTDYSLTISNLEQEDIATYFCQQGNTLPYTFGGGTKLEITGGGGGSGGGGSGGGGSEVKLQESGPGLVAPSQSLSVTCTVSGVSLPDYGVSWIRQPPRKGLEWLGVIWGSETTYYNSALKSRLTIIKDNSKSQVFLKMNSLQTDDTAIYYCAKHYYYGGSYAMDYWGQGTSVTVSSSPTSKETIGDYTWTNGSQPAVQPAVHLQAQIQIRVMYTTQGGGEAWGISVLNPNKTKVQGSAEGAHPHLLLSFPYGHLSFGFMQDLQQKVVYLSYMAVEYNVSFPHAAQWTFSAQNASLRDLQAPLGQSFSASNSSIILSPAVHLDLLSLRLQAAQLPHTGVFGQSFSAPSDRSAMGRRVFLLFAVLLLGFFIFTFLRVPETRGRTFDQISAAFRRTPSLLEQEVKPSTELEYLGPDENDG

SEQ ID NO: 53 - protein, 522 aa, synthetic construct
  REGION 1..522: note = Chimeric Antigen Receptor
MRPRLWLLLAAQLTVLHGNSVLEQKLISEEDLGGGGGGDIQMTQTTSSLSASLGDRVTISCRASQDISKYLNWYQQKPDGTVKLLIYHTSRLHSGVPSRFSGSGSGTDYSLTISNLEQEDIATYFCQQGNTLPYTFGGGTKLEITGGGGGSGGGGSGGGGSEVKLQESGPGLVAPSQSLSVTCTVSGVSLPDYGVSWIRQPPRKGLEWLGVIWGSETTYYNSALKSRLTIIKDNSKSQVFLKMNSLQTDDTAIYYCAKHYYYGGSYAMDYWGQGTSVTVSSSPTSKETIGDYTWTNGSQPAVQPAVHLQAQIQIRVMYTTQGGGEAWGISVLNPNKTKVQGSAEGAHPHLLLSFPYGHLSFGFMQDLQQKVVYLSYMAVEYNVSFPHAAQWTFSAQNASLRDLQAPLGQSFSASNSSIILSPAVHLDLLSLRLQAAQLPHTGVFGQSFSAPSDRSAMGPYVRRLFAVLLLGFFIFTFLRVPETRGRTFDQISAAFRRTPSLLEQEVKPSTELEYLGPDENDG

SEQ ID NO: 54 - protein, 522 aa, synthetic construct
  REGION 1..522: note = Chimeric Antigen Receptor
MRPRLWLLLAAQLTVLHGNSVLEQKLISEEDLGGGGGGDIQMTQTTSSLSASLGDRVTISCRASQDISKYLNWYQQKPDGTVKLLIYHTSRLHSGVPSRFSGSGSGTDYSLTISNLEQEDIATYFCQQGNTLPYTFGGGTKLEITGGGGGSGGGGSGGGGSEVKLQESGPGLVAPSQSLSVTCTVSGVSLPDYGVSWIRQPPRKGLEWLGVIWGSETTYYNSALKSRLTIIKDNSKSQVFLKMNSLQTDDTAIYYCAKHYYYGGSYAMDYWGQGTSVTVSSSPTSKETIGDYTWTNGSQPAVQPAVHLQAQIQIRVMYTTQGGGEAWGISVLNPNKTKVQGSAEGAHPHLLLSFPYGHLSFGFMQDLQQKVVYLSYMAVEYNVSFPHAAQWTFSAQNASLRDLQAPLGQSFSASNSSIILSPAVHLDLLSLRLQAAQLPHTGVFGQSFSAPSDRSAMGPYVFRRFAVLLLGFFIFTFLRVPETRGRTFDQISAAFRRTPSLLEQEVKPSTELEYLGPDENDG

SEQ ID NO: 55 - protein, 522 aa, synthetic construct
  REGION 1..522: note = Chimeric Antigen Receptor
MRPRLWLLLAAQLTVLHGNSVLEQKLISEEDLGGGGGGDIQMTQTTSSLSASLGDRVTISCRASQDISKYLNWYQQKPDGTVKLLIYHTSRLHSGVPSRFSGSGSGTDYSLTISNLEQEDIATYFCQQGNTLPYTFGGGTKLEITGGGGGSGGGGSGGGGSEVKLQESGPGLVAPSQSLSVTCTVSGVSLPDYGVSWIRQPPRKGLEWLGVIWGSETTYYNSALKSRLTIIKDNSKSQVFLKMNSLQTDDTAIYYCAKHYYYGGSYAMDYWGQGTSVTVSSSPTSKETIGDYTWTNGSQPAVQPAVHLQAQIQIRVMYTTQGGGEAWGISVLNPNKTKVQGSAEGAHPHLLLSFPYGHLSFGFMQDLQQKVVYLSYMAVEYNVSFPHAAQWTFSAQNASLRDLQAPLGQSFSASNSSIILSPAVHLDLLSLRLQAAQLPHTGVFGQSFSAPSDRSAMGPRRFRRFAVLLLGFFIFTFLRVPETRGRTFDQISAAFRRTPSLLEQEVKPSTELEYLGPDENDG

SEQ ID NO: 56 - protein, 522 aa, synthetic construct
  REGION 1..522: note = Chimeric Antigen Receptor
MRPRLWLLLAAQLTVLHGNSVLEQKLISEEDLGGGGGGDIQMTQTTSSLSASLGDRVTISCRASQDISKYLNWYQQKPDGTVKLLIYHTSRLHSGVPSRFSGSGSGTDYSLTISNLEQEDIATYFCQQGNTLPYTFGGGTKLEITGGGGGSGGGGSGGGGSEVKLQESGPGLVAPSQSLSVTCTVSGVSLPDYGVSWIRQPPRKGLEWLGVIWGSETTYYNSALKSRLTIIKDNSKSQVFLKMNSLQTDDTAIYYCAKHYYYGGSYAMDYWGQGTSVTVSSSPTSKETIGDYTWTNGSQPAVQPAVHLQAQIQIRVMYTTQGGGEAWGISVLNPNKTKVQGSAEGAHPHLLLSFPYGHLSFGFMQDLQQKVVYLSYMAVEYNVSFPHAAQWTFSAQNASLRDLQAPLGQSFSASNSSIILSPAVHLDLLSLRLQAAQLPHTGVFGQSFSAPSDRSAMGPYRRRRFAVLLLGFFIFTFLRVPETRGRTFDQISAAFRRTPSLLEQEVKPSTELEYLGPDENDG

SEQ ID NO: 57 - protein, 587 aa, synthetic construct
  REGION 1..587: note = Chimeric Antigen Receptor
MRPRLWLLLAAQLTVLHGNSVLEQKLISEEDLGGGGGGDIQMTQTTSSLSASLGDRVTISCRASQDISKYLNWYQQKPDGTVKLLIYHTSRLHSGVPSRFSGSGSGTDYSLTISNLEQEDIATYFCQQGNTLPYTFGGGTKLEITGGGGGSGGGGSGGGGSEVKLQESGPGLVAPSQSLSVTCTVSGVSLPDYGVSWIRQPPRKGLEWLGVIWGSETTYYNSALKSRLTIIKDNSKSQVFLKMNSLQTDDTAIYYCAKHYYYGGSYAMDYWGQGTSVTVSSSPTSKETIGDYTWTNGSQPAVQPAVHLQAQIQIRVMYTTQGGGEAWGISVLNPNKTKVQGSAEGAHPHLLLSFPYGHLSFGFMQDLQQKVVYLSYMAVEYNVSFPHAAQWTFSAQNASLRDLQAPLGQSFSASNSSIILSPAVHLDLLSLRLQAAQLPHTGVFGQSFSAPSDRSAMGPYVFLLFAVLLLGFFIFTFLCPESPRYLYIIQNLEGPARKSLKRLTGWADVSGVLAELKDEKRKLERERPLSLLQLLGSRTHRQPRVPETRGRTFDQISAAFRRTPSLLEQEVKPSTELEYLGPDENDG

SEQ ID NO: 58 - protein, 587 aa, synthetic construct
  REGION 1..587: note = Chimeric Antigen Receptor
MRPRLWLLLAAQLTVLHGNSVLEQKLISEEDLGGGGGGDIQMTQTTSSLSASLGDRVTISCRASQDISKYLNWYQQKPDGTVKLLIYHTSRLHSGVPSRFSGSGSGTDYSLTISNLEQEDIATYFCQQGNTLPYTFGGGTKLEITGGGGGSGGGGSGGGGSEVKLQESGPGLVAPSQSLSVTCTVSGVSLPDYGVSWIRQPPRKGLEWLGVIWGSETTYYNSALKSRLTIIKDNSKSQVFLKMNSLQTDDTAIYYCAKHYYYGGSYAMDYWGQGTSVTVSSSPTSKETIGDYTWTNGSQPAVQPAVHLQAQIQIRVMYTTQGGGEAWGISVLNPNKTKVQGSAEGAHPHLLLSFPYGHLSFGFMQDLQQKVVYLSYMAVEYNVSFPHAAQWTFSAQNASLRDLQAPLGQSFSASNSSIILSPAVHLDLLSLRLQAAQLPHTGVFGQSFSAPSDRSAMGPRVFLLFAVLLLGFFIFTFLCPESPRYLYIIQNLEGPARKSLKRLTGWADVSGVLAELKDEKRKLERERPLSLLQLLGSRTHRQPRVPETRGRTFDQISAAFRRTPSLLEQEVKPSTELEYLGPDENDG

SEQ ID NO: 59 - protein, 587 aa, synthetic construct
  REGION 1..587: note = Chimeric Antigen Receptor
MRPRLWLLLAAQLTVLHGNSVLEQKLISEEDLGGGGGGDIQMTQTTSSLSASLGDRVTISCRASQDISKYLNWYQQKPDGTVKLLIYHTSRLHSGVPSRFSGSGSGTDYSLTISNLEQEDIATYFCQQGNTLPYTFGGGTKLEITGGGGGSGGGGSGGGGSEVKLQESGPGLVAPSQSLSVTCTVSGVSLPDYGVSWIRQPPRKGLEWLGVIWGSETTYYNSALKSRLTIIKDNSKSQVFLKMNSLQTDDTAIYYCAKHYYYGGSYAMDYWGQGTSVTVSSSPTSKETIGDYTWTNGSQPAVQPAVHLQAQIQIRVMYTTQGGGEAWGISVLNPNKTKVQGSAEGAHPHLLLSFPYGHLSFGFMQDLQQKVVYLSYMAVEYNVSFPHAAQWTFSAQNASLRDLQAPLGQSFSASNSSIILSPAVHLDLLSLRLQAAQLPHTGVFGQSFSAPSDRSAMGPYRFLLFAVLLLGFFIFTFLCPESPRYLYIIQNLEGPARKSLKRLTGWADVSGVLAELKDEKRKLERERPLSLLQLLGSRTHRQPRVPETRGRTFDQISAAFRRTPSLLEQEVKPSTELEYLGPDENDG

SEQ ID NO: 60 - protein, 587 aa, synthetic construct
  REGION 1..587: note = Chimeric Antigen Receptor
MRPRLWLLLAAQLTVLHGNSVLEQKLISEEDLGGGGGGDIQMTQTTSSLSASLGDRVTISCRASQDISKYLNWYQQKPDGTVKLLIYHTSRLHSGVPSRFSGSGSGTDYSLTISNLEQEDIATYFCQQGNTLPYTFGGGTKLEITGGGGGSGGGGSGGGGSEVKLQESGPGLVAPSQSLSVTCTVSGVSLPDYGVSWIRQPPRKGLEWLGVIWGSETTYYNSALKSRLTIIKDNSKSQVFLKMNSLQTDDTAIYYCAKHYYYGGSYAMDYWGQGTSVTVSSSPTSKETIGDYTWTNGSQPAVQPAVHLQAQIQIRVMYTTQGGGEAWGISVLNPNKTKVQGSAEGAHPHLLLSFPYGHLSFGFMQDLQQKVVYLSYMAVEYNVSFPHAAQWTFSAQNASLRDLQAPLGQSFSASNSSIILSPAVHLDLLSLRLQAAQLPHTGVFGQSFSAPSDRSAMGRRVFLLFAVLLLGFFIFTFLCPESPRYLYIIQNLEGPARKSLKRLTGWADVSGVLAELKDEKRKLERERPLSLLQLLGSRTHRQPRVPETRGRTFDQISAAFRRTPSLLEQEVKPSTELEYLGPDENDG

SEQ ID NO: 61 - protein, 587 aa, synthetic construct
  REGION 1..587: note = Chimeric Antigen Receptor
MRPRLWLLLAAQLTVLHGNSVLEQKLISEEDLGGGGGGDIQMTQTTSSLSASLGDRVTISCRASQDISKYLNWYQQKPDGTVKLLIYHTSRLHSGVPSRFSGSGSGTDYSLTISNLEQEDIATYFCQQGNTLPYTFGGGTKLEITGGGGGSGGGGSGGGGSEVKLQESGPGLVAPSQSLSVTCTVSGVSLPDYGVSWIRQPPRKGLEWLGVIWGSETTYYNSALKSRLTIIKDNSKSQVFLKMNSLQTDDTAIYYCAKHYYYGGSYAMDYWGQGTSVTVSSSPTSKETIGDYTWTNGSQPAVQPAVHLQAQIQIRVMYTTQGGGEAWGISVLNPNKTKVQGSAEGAHPHLLLSFPYGHLSFGFMQDLQQKVVYLSYMAVEYNVSFPHAAQWTFSAQNASLRDLQAPLGQSFSASNSSIILSPAVHLDLLSLRLQAAQLPHTGVFGQSFSAPSDRSAMGPYVRRLFAVLLLGFFIFTFLCPESPRYLYIIQNLEGPARKSLKRLTGWADVSGVLAELKDEKRKLERERPLSLLQLLGSRTHRQPRVPETRGRTFDQISAAFRRTPSLLEQEVKPSTELEYLGPDENDG

SEQ ID NO: 62 - protein, 587 aa, synthetic construct
  REGION 1..587: note = Chimeric Antigen Receptor
MRPRLWLLLAAQLTVLHGNSVLEQKLISEEDLGGGGGGDIQMTQTTSSLSASLGDRVTISCRASQDISKYLNWYQQKPDGTVKLLIYHTSRLHSGVPSRFSGSGSGTDYSLTISNLEQEDIATYFCQQGNTLPYTFGGGTKLEITGGGGGSGGGGSGGGGSEVKLQESGPGLVAPSQSLSVTCTVSGVSLPDYGVSWIRQPPRKGLEWLGVIWGSETTYYNSALKSRLTIIKDNSKSQVFLKMNSLQTDDTAIYYCAKHYYYGGSYAMDYWGQGTSVTVSSSPTSKETIGDYTWTNGSQPAVQPAVHLQAQIQIRVMYTTQGGGEAWGISVLNPNKTKVQGSAEGAHPHLLLSFPYGHLSFGFMQDLQQKVVYLSYMAVEYNVSFPHAAQWTFSAQNASLRDLQAPLGQSFSASNSSIILSPAVHLDLLSLRLQAAQLPHTGVFGQSFSAPSDRSAMGPYVFRRFAVLLLGFFIFTFLCPESPRYLYIIQNLEGPARKSLKRLTGWADVSGVLAELKDEKRKLERERPLSLLQLLGSRTHRQPRVPETRGRTFDQISAAFRRTPSLLEQEVKPSTELEYLGPDENDG

SEQ ID NO: 63 - protein, 587 aa, synthetic construct
  REGION 1..587: note = Chimeric Antigen Receptor
MRPRLWLLLAAQLTVLHGNSVLEQKLISEEDLGGGGGGDIQMTQTTSSLSASLGDRVTISCRASQDISKYLNWYQQKPDGTVKLLIYHTSRLHSGVPSRFSGSGSGTDYSLTISNLEQEDIATYFCQQGNTLPYTFGGGTKLEITGGGGGSGGGGSGGGGSEVKLQESGPGLVAPSQSLSVTCTVSGVSLPDYGVSWIRQPPRKGLEWLGVIWGSETTYYNSALKSRLTIIKDNSKSQVFLKMNSLQTDDTAIYYCAKHYYYGGSYAMDYWGQGTSVTVSSSPTSKETIGDYTWTNGSQPAVQPAVHLQAQIQIRVMYTTQGGGEAWGISVLNPNKTKVQGSAEGAHPHLLLSFPYGHLSFGFMQDLQQKVVYLSYMAVEYNVSFPHAAQWTFSAQNASLRDLQAPLGQSFSASNSSIILSPAVHLDLLSLRLQAAQLPHTGVFGQSFSAPSDRSAMGPRRFLLFAVLLLGFFIFTFLCPESPRYLYIIQNLEGPARKSLKRLTGWADVSGVLAELKDEKRKLERERPLSLLQLLGSRTHRQPRVPETRGRTFDQISAAFRRTPSLLEQEVKPSTELEYLGPDENDG

SEQ ID NO: 64 - protein, 587 aa, synthetic construct
  REGION 1..587: note = Chimeric Antigen Receptor
MRPRLWLLLAAQLTVLHGNSVLEQKLISEEDLGGGGGGDIQMTQTTSSLSASLGDRVTISCRASQDISKYLNWYQQKPDGTVKLLIYHTSRLHSGVPSRFSGSGSGTDYSLTISNLEQEDIATYFCQQGNTLPYTFGGGTKLEITGGGGGSGGGGSGGGGSEVKLQESGPGLVAPSQSLSVTCTVSGVSLPDYGVSWIRQPPRKGLEWLGVIWGSETTYYNSALKSRLTIIKDNSKSQVFLKMNSLQTDDTAIYYCAKHYYYGGSYAMDYWGQGTSVTVSSSPTSKETIGDYTWTNGSQPAVQPAVHLQAQIQIRVMYTTQGGGEAWGISVLNPNKTKVQGSAEGAHPHLLLSFPYGHLSFGFMQDLQQKVVYLSYMAVEYNVSFPHAAQWTFSAQNASLRDLQAPLGQSFSASNSSIILSPAVHLDLLSLRLQAAQLPHTGVFGQSFSAPSDRSAMGPYRRLLFAVLLLGFFIFTFLCPESPRYLYIIQNLEGPARKSLKRLTGWADVSGVLAELKDEKRKLERERPLSLLQLLGSRTHRQPRVPETRGRTFDQISAAFRRTPSLLEQEVKPSTELEYLGPDENDG

SEQ ID NO: 65 - protein, 22 aa, synthetic construct
  REGION 1..22: note = signal peptide
MRPRLWLLLAAQLTVLHGNSVL

SEQ ID NO: 66 - DNA, 1761 bp, synthetic construct
  misc_feature 1..1761: note = DNA code of SEQ ID No 57
  source 1..1761: mol_type = other DNA
atgagacctaggttgtggctgttgctcgcagcccaattgactgtactccacggtaacagcgtattggaacaaaaacttattagcgaagaggatcttggaggcggtggaggtggggatatacaaatgacacagacgacttcctccctctccgcaagtcttggggatcgggtaactatctcatgccgggcgtcccaagacatttcaaagtacctgaactggtatcaacaaaaacctgatggaacagtcaaactcctcatatatcacaccagcagactccattccggggtgcctagccgcttcagcgggagtggttccggaacagactatagtcttacaataagtaacctggaacaggaagatattgccacttacttctgtcagcagggcaatacactcccatatacatttggaggtggcacgaaacttgaaatcaccggtggaggaggcggctctggaggtggcggctcaggtggtggtggttctgaggtaaaacttcaggagtcaggaccaggacttgtagctcccagccaatccttgagtgtcacatgcacagtatctggggtctcacttcctgactatggcgtttcatggataagacaaccaccccgaaaaggtttggagtggctgggtgtgatttggggttctgagaccacttactacaatagcgcgttgaagtccaggcttactattattaaagacaattccaagtctcaagtcttcctgaagatgaattcacttcaaactgatgatactgcgatatattattgtgccaagcactattactacggtgggtcctacgctatggattactggggacagggcacctcagtaaccgtatcctcctcccctacctccaaggaaaccatcggagattatacctggaccaacggatcccagccttgtgtgcaaccttgcgtccatctgcaggcgcaaatacaaatccgggtgatgtacaccacgcaagggggaggcgaagcgtggggcattagtgtcttgaacccaaataagactaaggttcaggggagctgcgagggggcacatccacatcttctcctctcttttccttatggccatttgtcatttggatttatgcaggacttgcaacaaaaggtcgtctatttgtcctatatggccgttgagtacaatgtctctttcccccatgctgcccaatggaccttcagtgcgcagaacgcgagtctccgagatctgcaggctcccttgggtcaaagtttcagctgctcaaatagtagtatcatactgtcccccgcggtacacctcgatcttcttagtctccggctgcaggccgctcaacttcctcacactggcgtattcggccagagcttttcctgtcctagtgaccgcagcgcgatgggcccttatgtgtttctgttgttcgcggtacttttgctgggcttctttatttttaccttcttgtgccctgagagccctagatacctgtacatcatccagaacctggagggccctgctagaaagagcctgaagagactgaccggctgggctgacgtgagcggcgtgctggctgagctgaaggacgagaagagaaagctggagagagagagacctctgagcctgctgcagctgctgggcagcagaacccacagacagcctcgcgtgcccgagactcgagggcggacttttgaccagatttctgcagctttccgacgaacaccatccctgctcgaacaggaagtcaaacctagtacggaactggaatacttggggcccgacgaaaacgacgga

SEQ ID NO: 67 - DNA, 1761 bp, synthetic construct
  misc_feature 1..1761: note = DNA code of SEQ ID No 58
  source 1..1761: mol_type = other DNA
atgagacctaggttgtggctgttgctcgcagcccaattgactgtactccacggtaacagcgtattggaacaaaaacttattagcgaagaggatcttggaggcggtggaggtggggatatacaaatgacacagacgacttcctccctctccgcaagtcttggggatcgggtaactatctcatgccgggcgtcccaagacatttcaaagtacctgaactggtatcaacaaaaacctgatggaacagtcaaactcctcatatatcacaccagcagactccattccggggtgcctagccgcttcagcgggagtggttccggaacagactatagtcttacaataagtaacctggaacaggaagatattgccacttacttctgtcagcagggcaatacactcccatatacatttggaggtggcacgaaacttgaaatcaccggtggaggaggcggctctggaggtggcggctcaggtggtggtggttctgaggtaaaacttcaggagtcaggaccaggacttgtagctcccagccaatccttgagtgtcacatgcacagtatctggggtctcacttcctgactatggcgtttcatggataagacaaccaccccgaaaaggtttggagtggctgggtgtgatttggggttctgagaccacttactacaatagcgcgttgaagtccaggcttactattattaaagacaattccaagtctcaagtcttcctgaagatgaattcacttcaaactgatgatactgcgatatattattgtgccaagcactattactacggtgggtcctacgctatggattactggggacagggcacctcagtaaccgtatcctcctcccctacctccaaggaaaccatcggagattatacctggaccaacggatcccagccttgtgtgcaaccttgcgtccatctgcaggcgcaaatacaaatccgggtgatgtacaccacgcaagggggaggcgaagcgtggggcattagtgtcttgaacccaaataagactaaggttcaggggagctgcgagggggcacatccacatcttctcctctcttttccttatggccatttgtcatttggatttatgcaggacttgcaacaaaaggtcgtctatttgtcctatatggccgttgagtacaatgtctctttcccccatgctgcccaatggaccttcagtgcgcagaacgcgagtctccgagatctgcaggctcccttgggtcaaagtttcagctgctcaaatagtagtatcatactgtcccccgcggtacacctcgatcttcttagtctccggctgcaggccgctcaacttcctcacactggcgtattcggccagagcttttcctgtcctagtgaccgcagcgcgatgggccctagagtgtttctgttgttcgcggtacttttgctgggcttctttatttttaccttcttgtgccctgagagccctagatacctgtacatcatccagaacctggagggccctgctagaaagagcctgaagagactgaccggctgggctgacgtgagcggcgtgctggctgagctgaaggacgagaagagaaagctggagagagagagacctctgagcctgctgcagctgctgggcagcagaacccacagacagcctcgcgtgcccgagactcgagggcggacttttgaccagatttctgcagctttccgacgaacaccatccctgctcgaacaggaagtcaaacctagtacggaactggaatacttggggcccgacgaaaacgacgga

SEQ ID NO: 68 - skipped

SEQ ID NO: 69 - DNA, 1761 bp, synthetic construct
  misc_feature 1..1761: note = DNA code of SEQ ID No 60
  source 1..1761: mol_type = other DNA
atgagacctaggttgtggctgttgctcgcagcccaattgactgtactccacggtaacagcgtattggaacaaaaacttattagcgaagaggatcttggaggcggtggaggtggggatatacaaatgacacagacgacttcctccctctccgcaagtcttggggatcgggtaactatctcatgccgggcgtcccaagacatttcaaagtacctgaactggtatcaacaaaaacctgatggaacagtcaaactcctcatatatcacaccagcagactccattccggggtgcctagccgcttcagcgggagtggttccggaacagactatagtcttacaataagtaacctggaacaggaagatattgccacttacttctgtcagcagggcaatacactcccatatacatttggaggtggcacgaaacttgaaatcaccggtggaggaggcggctctggaggtggcggctcaggtggtggtggttctgaggtaaaacttcaggagtcaggaccaggacttgtagctcccagccaatccttgagtgtcacatgcacagtatctggggtctcacttcctgactatggcgtttcatggataagacaaccaccccgaaaaggtttggagtggctgggtgtgatttggggttctgagaccacttactacaatagcgcgttgaagtccaggcttactattattaaagacaattccaagtctcaagtcttcctgaagatgaattcacttcaaactgatgatactgcgatatattattgtgccaagcactattactacggtgggtcctacgctatggattactggggacagggcacctcagtaaccgtatcctcctcccctacctccaaggaaaccatcggagattatacctggaccaacggatcccagccttgtgtgcaaccttgcgtccatctgcaggcgcaaatacaaatccgggtgatgtacaccacgcaagggggaggcgaagcgtggggcattagtgtcttgaacccaaataagactaaggttcaggggagctgcgagggggcacatccacatcttctcctctcttttccttatggccatttgtcatttggatttatgcaggacttgcaacaaaaggtcgtctatttgtcctatatggccgttgagtacaatgtctctttcccccatgctgcccaatggaccttcagtgcgcagaacgcgagtctccgagatctgcaggctcccttgggtcaaagtttcagctgctcaaatagtagtatcatactgtcccccgcggtacacctcgatcttcttagtctccggctgcaggccgctcaacttcctcacactggcgtattcggccagagcttttcctgtcctagtgaccgcagcgcgatgggcagaagagtgtttctgttgttcgcggtacttttgctgggcttctttatttttaccttcttgtgccctgagagccctagatacctgtacatcatccagaacctggagggccctgctagaaagagcctgaagagactgaccggctgggctgacgtgagcggcgtgctggctgagctgaaggacgagaagagaaagctggagagagagagacctctgagcctgctgcagctgctgggcagcagaacccacagacagcctcgcgtgcccgagactcgagggcggacttttgaccagatttctgcagctttccgacgaacaccatccctgctcgaacaggaagtcaaacctagtacggaactggaatacttggggcccgacgaaaacgacgga

SEQ ID NO: 70 - DNA, 1761 bp, synthetic construct
  misc_feature 1..1761: note = DNA code of SEQ ID No 61
  source 1..1761: mol_type = other DNA
atgagacctaggttgtggctgttgctcgcagcccaattgactgtactccacggtaacagcgtattggaacaaaaacttattagcgaagaggatcttggaggcggtggaggtggggatatacaaatgacacagacgacttcctccctctccgcaagtcttggggatcgggtaactatctcatgccgggcgtcccaagacatttcaaagtacctgaactggtatcaacaaaaacctgatggaacagtcaaactcctcatatatcacaccagcagactccattccggggtgcctagccgcttcagcgggagtggttccggaacagactatagtcttacaataagtaacctggaacaggaagatattgccacttacttctgtcagcagggcaatacactcccatatacatttggaggtggcacgaaacttgaaatcaccggtggaggaggcggctctggaggtggcggctcaggtggtggtggttctgaggtaaaacttcaggagtcaggaccaggacttgtagctcccagccaatccttgagtgtcacatgcacagtatctggggtctcacttcctgactatggcgtttcatggataagacaaccaccccgaaaaggtttggagtggctgggtgtgatttggggttctgagaccacttactacaatagcgcgttgaagtccaggcttactattattaaagacaattccaagtctcaagtcttcctgaagatgaattcacttcaaactgatgatactgcgatatattattgtgccaagcactattactacggtgggtcctacgctatggattactggggacagggcacctcagtaaccgtatcctcctcccctacctccaaggaaaccatcggagattatacctggaccaacggatcccagccttgtgtgcaaccttgcgtccatctgcaggcgcaaatacaaatccgggtgatgtacaccacgcaagggggaggcgaagcgtggggcattagtgtcttgaacccaaataagactaaggttcaggggagctgcgagggggcacatccacatcttctcctctcttttccttatggccatttgtcatttggatttatgcaggacttgcaacaaaaggtcgtctatttgtcctatatggccgttgagtacaatgtctctttcccccatgctgcccaatggaccttcagtgcgcagaacgcgagtctccgagatctgcaggctcccttgggtcaaagtttcagctgctcaaatagtagtatcatactgtcccccgcggtacacctcgatcttcttagtctccggctgcaggccgctcaacttcctcacactggcgtattcggccagagcttttcctgtcctagtgaccgcagcgcgatgggcccttatgtgagaagattgttcgcggtacttttgctgggcttctttatttttaccttcttgtgccctgagagccctagatacctgtacatcatccagaacctggagggccctgctagaaagagcctgaagagactgaccggctgggctgacgtgagcggcgtgctggctgagctgaaggacgagaagagaaagctggagagagagagacctctgagcctgctgcagctgctgggcagcagaacccacagacagcctcgcgtgcccgagactcgagggcggacttttgaccagatttctgcagctttccgacgaacaccatccctgctcgaacaggaagtcaaacctagtacggaactggaatacttggggcccgacgaaaacgacgga

SEQ ID NO: 71 - DNA, 1761 bp, synthetic construct
  misc_feature 1..1761: note = DNA code of SEQ ID No 62
  source 1..1761: mol_type = other DNA
atgagacctaggttgtggctgttgctcgcagcccaattgactgtactccacggtaacagcgtattggaacaaaaacttattagcgaagaggatcttggaggcggtggaggtggggatatacaaatgacacagacgacttcctccctctccgcaagtcttggggatcgggtaactatctcatgccgggcgtcccaagacatttcaaagtacctgaactggtatcaacaaaaacctgatggaacagtcaaactcctcatatatcacaccagcagactccattccggggtgcctagccgcttcagcgggagtggttccggaacagactatagtcttacaataagtaacctggaacaggaagatattgccacttacttctgtcagcagggcaatacactcccatatacatttggaggtggcacgaaacttgaaatcaccggtggaggaggcggctctggaggtggcggctcaggtggtggtggttctgaggtaaaacttcaggagtcaggaccaggacttgtagctcccagccaatccttgagtgtcacatgcacagtatctggggtctcacttcctgactatggcgtttcatggataagacaaccaccccgaaaaggtttggagtggctgggtgtgatttggggttctgagaccacttactacaatagcgcgttgaagtccaggcttactattattaaagacaattccaagtctcaagtcttcctgaagatgaattcacttcaaactgatgatactgcgatatattattgtgccaagcactattactacggtgggtcctacgctatggattactggggacagggcacctcagtaaccgtatcctcctcccctacctccaaggaaaccatcggagattatacctggaccaacggatcccagccttgtgtgcaaccttgcgtccatctgcaggcgcaaatacaaatccgggtgatgtacaccacgcaagggggaggcgaagcgtggggcattagtgtcttgaacccaaataagactaaggttcaggggagctgcgagggggcacatccacatcttctcctctcttttccttatggccatttgtcatttggatttatgcaggacttgcaacaaaaggtcgtctatttgtcctatatggccgttgagtacaatgtctctttcccccatgctgcccaatggaccttcagtgcgcagaacgcgagtctccgagatctgcaggctcccttgggtcaaagtttcagctgctcaaatagtagtatcatactgtcccccgcggtacacctcgatcttcttagtctccggctgcaggccgctcaacttcctcacactggcgtattcggccagagcttttcctgtcctagtgaccgcagcgcgatgggcccttatgtgtttagaagattcgcggtacttttgctgggcttctttatttttaccttcttgtgccctgagagccctagatacctgtacatcatccagaacctggagggccctgctagaaagagcctgaagagactgaccggctgggctgacgtgagcggcgtgctggctgagctgaaggacgagaagagaaagctggagagagagagacctctgagcctgctgcagctgctgggcagcagaacccacagacagcctcgcgtgcccgagactcgagggcggacttttgaccagatttctgcagctttccgacgaacaccatccctgctcgaacaggaagtcaaacctagtacggaactggaatacttggggcccgacgaaaacgacgga

SEQ ID NO: 72 - DNA, 1761 bp, synthetic construct
  misc_feature 1..1761: note = DNA code of SEQ ID No 63
  source 1..1761: mol_type = other DNA
atgagacctaggttgtggctgttgctcgcagcccaattgactgtactccacggtaacagcgtattggaacaaaaacttattagcgaagaggatcttggaggcggtggaggtggggatatacaaatgacacagacgacttcctccctctccgcaagtcttggggatcgggtaactatctcatgccgggcgtcccaagacatttcaaagtacctgaactggtatcaacaaaaacctgatggaacagtcaaactcctcatatatcacaccagcagactccattccggggtgcctagccgcttcagcgggagtggttccggaacagactatagtcttacaataagtaacctggaacaggaagatattgccacttacttctgtcagcagggcaatacactcccatatacatttggaggtggcacgaaacttgaaatcaccggtggaggaggcggctctggaggtggcggctcaggtggtggtggttctgaggtaaaacttcaggagtcaggaccaggacttgtagctcccagccaatccttgagtgtcacatgcacagtatctggggtctcacttcctgactatggcgtttcatggataagacaaccaccccgaaaaggtttggagtggctgggtgtgatttggggttctgagaccacttactacaatagcgcgttgaagtccaggcttactattattaaagacaattccaagtctcaagtcttcctgaagatgaattcacttcaaactgatgatactgcgatatattattgtgccaagcactattactacggtgggtcctacgctatggattactggggacagggcacctcagtaaccgtatcctcctcccctacctccaaggaaaccatcggagattatacctggaccaacggatcccagccttgtgtgcaaccttgcgtccatctgcaggcgcaaatacaaatccgggtgatgtacaccacgcaagggggaggcgaagcgtggggcattagtgtcttgaacccaaataagactaaggttcaggggagctgcgagggggcacatccacatcttctcctctcttttccttatggccatttgtcatttggatttatgcaggacttgcaacaaaaggtcgtctatttgtcctatatggccgttgagtacaatgtctctttcccccatgctgcccaatggaccttcagtgcgcagaacgcgagtctccgagatctgcaggctcccttgggtcaaagtttcagctgctcaaatagtagtatcatactgtcccccgcggtacacctcgatcttcttagtctccggctgcaggccgctcaacttcctcacactggcgtattcggccagagcttttcctgtcctagtgaccgcagcgcgatgggccctagaagatttctgttgttcgcggtacttttgctgggcttctttatttttaccttcttgtgccctgagagccctagatacctgtacatcatccagaacctggagggccctgctagaaagagcctgaagagactgaccggctgggctgacgtgagcggcgtgctggctgagctgaaggacgagaagagaaagctggagagagagagacctctgagcctgctgcagctgctgggcagcagaacccacagacagcctcgcgtgcccgagactcgagggcggacttttgaccagatttctgcagctttccgacgaacaccatccctgctcgaacaggaagtcaaacctagtacggaactggaatacttggggcccgacgaaaacgacgga

SEQ ID NO: 73 - DNA, 1761 bp, synthetic construct
  misc_feature 1..1761: note = DNA code of SEQ ID No 64
  source 1..1761: mol_type = other DNA
atgagacctaggttgtggctgttgctcgcagcccaattgactgtactccacggtaacagcgtattggaacaaaaacttattagcgaagaggatcttggaggcggtggaggtggggatatacaaatgacacagacgacttcctccctctccgcaagtcttggggatcgggtaactatctcatgccgggcgtcccaagacatttcaaagtacctgaactggtatcaacaaaaacctgatggaacagtcaaactcctcatatatcacaccagcagactccattccggggtgcctagccgcttcagcgggagtggttccggaacagactatagtcttacaataagtaacctggaacaggaagatattgccacttacttctgtcagcagggcaatacactcccatatacatttggaggtggcacgaaacttgaaatcaccggtggaggaggcggctctggaggtggcggctcaggtggtggtggttctgaggtaaaacttcaggagtcaggaccaggacttgtagctcccagccaatccttgagtgtcacatgcacagtatctggggtctcacttcctgactatggcgtttcatggataagacaaccaccccgaaaaggtttggagtggctgggtgtgatttggggttctgagaccacttactacaatagcgcgttgaagtccaggcttactattattaaagacaattccaagtctcaagtcttcctgaagatgaattcacttcaaactgatgatactgcgatatattattgtgccaagcactattactacggtgggtcctacgctatggattactggggacagggcacctcagtaaccgtatcctcctcccctacctccaaggaaaccatcggagattatacctggaccaacggatcccagccttgtgtgcaaccttgcgtccatctgcaggcgcaaatacaaatccgggtgatgtacaccacgcaagggggaggcgaagcgtggggcattagtgtcttgaacccaaataagactaaggttcaggggagctgcgagggggcacatccacatcttctcctctcttttccttatggccatttgtcatttggatttatgcaggacttgcaacaaaaggtcgtctatttgtcctatatggccgttgagtacaatgtctctttcccccatgctgcccaatggaccttcagtgcgcagaacgcgagtctccgagatctgcaggctcccttgggtcaaagtttcagctgctcaaatagtagtatcatactgtcccccgcggtacacctcgatcttcttagtctccggctgcaggccgctcaacttcctcacactggcgtattcggccagagcttttcctgtcctagtgaccgcagcgcgatgggcccttatagaagactgttgttcgcggtacttttgctgggcttctttatttttaccttcttgtgccctgagagccctagatacctgtacatcatccagaacctggagggccctgctagaaagagcctgaagagactgaccggctgggctgacgtgagcggcgtgctggctgagctgaaggacgagaagagaaagctggagagagagagacctctgagcctgctgcagctgctgggcagcagaacccacagacagcctcgcgtgcccgagactcgagggcggacttttgaccagatttctgcagctttccgacgaacaccatccctgctcgaacaggaagtcaaacctagtacggaactggaatacttggggcccgacgaaaacgacgga